European Patent Specification EP 3 402 904 B1, published July 23, 2025. Title: SYNTHESIZING BARCODING SEQUENCES UTILIZING PHASE-SHIFT BLOCKS AND USES THEREOF. Applicant: Bio-Rad Laboratories, Inc. Application PCT/US2017/013205. The sequence listing filed with the application follows.

SEQUENCE LISTING (118 sequences)

SEQ ID NO: 1 - DNA, 62 bp, Artificial Sequence
  synthetic polynucleotide
  misc_feature (15)..(20): n = any nucleotide
  misc_feature (36)..(41): n = any nucleotide
  misc_feature (57)..(62): n = any nucleotide
cgctcttccgatctnnnnnngtgcgctgatcggagnnnnnntcggcatgtctggctnnnnnn

SEQ ID NO: 2 - DNA, 63 bp, Artificial Sequence
  synthetic polynucleotide
  misc_feature (16)..(21): n = any nucleotide
  misc_feature (37)..(42): n = any nucleotide
  misc_feature (58)..(63): n = any nucleotide
cgctcttccgatctannnnnngtgcgctgatcggagnnnnnntcggcatgtctggctnnnnnn

SEQ ID NO: 3 - DNA, 64 bp, Artificial Sequence
  synthetic polynucleotide
  misc_feature (17)..(22): n = any nucleotide
  misc_feature (38)..(43): n = any nucleotide
  misc_feature (59)..(64): n = any nucleotide
cgctcttccgatctcannnnnngtgcgctgatcggagnnnnnntcggcatgtctggctnnnnnn

SEQ ID NO: 4 - DNA, 65 bp, Artificial Sequence
  synthetic polynucleotide
  misc_feature (18)..(23): n = any nucleotide
  misc_feature (39)..(44): n = any nucleotide
  misc_feature (60)..(65): n = any nucleotide
cgctcttccgatctgcannnnnngtgcgctgatcggagnnnnnntcggcatgtctggctnnnnnn

SEQ ID NO: 5 - DNA, 66 bp, Artificial Sequence
  synthetic polynucleotide
  misc_feature (19)..(24): n = any nucleotide
  misc_feature (40)..(45): n = any nucleotide
  misc_feature (61)..(66): n = any nucleotide
cgctcttccgatcttgcannnnnngtgcgctgatcggagnnnnnntcggcatgtctggctnnnnnn

SEQ ID NO: 6 - DNA, 16 bp, Artificial Sequence
  synthetic oligonucleotide
cgtactctgcgttgat

SEQ ID NO: 7 - DNA, 15 bp, Artificial Sequence
  synthetic oligonucleotide
gcaatgcgatggcta

SEQ ID NO: 8 - DNA, 15 bp, Artificial Sequence
  synthetic oligonucleotide
ttcagctcagtggta

SEQ ID NO: 9 - DNA, 17 bp, Artificial Sequence
  synthetic oligonucleotide
  misc_feature (1)..(6): n = any nucleotide
  misc_feature (10)..(17): n = any nucleotide
nnnnnncgtnnnnnnnn

SEQ ID NO: 10 - DNA, 21 bp, Artificial Sequence
  synthetic oligonucleotide
baaaaaaaaaaaaaaaaaaaa

SEQ ID NO: 11 - DNA, 54 bp, Artificial Sequence
  synthetic polynucleotide
tttttttuuuctacacgcctgtccgcggaagcagtggtatcaacgcagagtacg

SEQ ID NO: 12 - DNA, 38 bp, Artificial Sequence
  synthetic polynucleotide
  misc_feature (16)..(21): n = any nucleotide
gcaatgcgatggctannnnnnacgtactctgcgttgat

SEQ ID NO: 13 - DNA, 39 bp, Artificial Sequence
  synthetic polynucleotide
  misc_feature (16)..(21): n = any nucleotide
gcaatgcgatggctannnnnnaccgtactctgcgttgat

SEQ ID NO: 14 - DNA, 40 bp, Artificial Sequence
  synthetic polynucleotide
  misc_feature (16)..(21): n = any nucleotide
gcaatgcgatggctannnnnnacgcgtactctgcgttgat

SEQ ID NO: 15 - DNA, 41 bp, Artificial Sequence
  synthetic polynucleotide
  misc_feature (16)..(21): n = any nucleotide
gcaatgcgatggctannnnnnacgtcgtactctgcgttgat

SEQ ID NO: 16 - DNA, 76 bp, Artificial Sequence
  synthetic polynucleotide
  misc_feature (56)..(61): n = any nucleotide
tttttttuuuctacacgcctgtccgcggaagcagtggtatcaacgcagagtacgtnnnnnntagccatcgcattgc

SEQ ID NO: 17 - DNA, 48 bp, Artificial Sequence
  synthetic polynucleotide
  misc_feature (16)..(21): n = any nucleotide
gcaatgcgatggctannnnnnacgtactctgcgttgataccactgctt

SEQ ID NO: 18 - DNA, 36 bp, Artificial Sequence
  synthetic polynucleotide
  misc_feature (16)..(21): n = any nucleotide
ttcagctcagtggtannnnnngcaatgcgatggcta

SEQ ID NO: 19 - DNA, 97 bp, Artificial Sequence
  synthetic polynucleotide
  misc_feature (56)..(61): n = any nucleotide
  misc_feature (77)..(82): n = any nucleotide
tttttttuuuctacacgcctgtccgcggaagcagtggtatcaacgcagagtacgtnnnnnntagccatcgcattgcnnnnnntaccactgagctgaa

SEQ ID NO: 20 - DNA, 53 bp, Artificial Sequence
  synthetic polynucleotide
  misc_feature (22)..(29): n = any nucleotide
  misc_feature (33)..(38): n = any nucleotide
baaaaaaaaaaaaaaaaaaaannnnnnnncgtnnnnnnttcagctcagtggta

SEQ ID NO: 21 - DNA, 95 bp, Artificial Sequence
  synthetic polynucleotide
  misc_feature (13)..(18): n = any nucleotide
  misc_feature (34)..(39): n = any nucleotide
  misc_feature (55)..(60): n = any nucleotide
  misc_feature (64)..(71): n = any nucleotide
cgcagagtacgtnnnnnntagccatcgcattgcnnnnnntaccactgagctgaannnnnnacgnnnnnnnnacgttttttttttttttttttttv

SEQ ID NO: 22 - DNA, 144 bp, Artificial Sequence
  synthetic polynucleotide
  misc_feature (55)..(55): n = a
  misc_feature (56)..(56): n = c or absent
  misc_feature (57)..(57): n =  g or absent if nucleotide in position 56 is absent
  misc_feature (58)..(58): n= t or absent if nucleotides in position 56 and 57 are absent
  misc_feature (60)..(65): n = any nucleotide
  misc_feature (81)..(86): n = any nucleotide
  misc_feature (102)..(109): n = any nucleotide
  misc_feature (113)..(120): n = any nucleotide
tttttttuuuctacacgcctgtccgcggaagcagtggtatcaacgcagagtacgnnnntnnnnnntagccatcgcattgcnnnnnntaccactgagctgaannnnnnnnacgnnnnnnnntgcaaaaaaaaaaaaaaaaaaaab

SEQ ID NO: 23 - DNA, 37 bp, Artificial Sequence
  synthetic polynucleotide
  misc_feature (17)..(22): n = any nucleotide
tagttgcgtctcatgcnnnnnnatcggtagcgtaacg

SEQ ID NO: 24 - DNA, 37 bp, Artificial Sequence; identical to SEQ ID NO: 23
  synthetic polynucleotide
  misc_feature (17)..(22): n = any nucleotide

SEQ ID NO: 25 - DNA, 37 bp, Artificial Sequence; identical to SEQ ID NO: 23
  synthetic polynucleotide
  misc_feature (17)..(22): n = any nucleotide

SEQ ID NO: 26 - DNA, 37 bp, Artificial Sequence
  synthetic polynucleotide
  misc_feature (17)..(22): n = any nucleotide
tagttgcgtctcatgcnnnnnngcatgcgttactgga

SEQ ID NO: 27 - DNA, 37 bp, Artificial Sequence; identical to SEQ ID NO: 26
  synthetic polynucleotide
  misc_feature (17)..(22): n = any nucleotide

SEQ ID NO: 28 - DNA, 37 bp, Artificial Sequence; identical to SEQ ID NO: 26
  synthetic polynucleotide
  misc_feature (17)..(22): n = any nucleotide

SEQ ID NO: 29 - DNA, 37 bp, Artificial Sequence
  synthetic polynucleotide
  misc_feature (17)..(22): n = any nucleotide
tagttgcgtctcatgcnnnnnncgtatagcgtagttc

SEQ ID NO: 30 - DNA, 37 bp, Artificial Sequence; identical to SEQ ID NO: 29
  synthetic polynucleotide
  misc_feature (17)..(22): n = any nucleotide

SEQ ID NO: 31 - DNA, 37 bp, Artificial Sequence; identical to SEQ ID NO: 29
  synthetic polynucleotide
  misc_feature (17)..(22): n = any nucleotide

SEQ ID NO: 32 - DNA, 36 bp, Artificial Sequence
  synthetic polynucleotide
  misc_feature (16)..(21): n = any nucleotide
tagccatcgcattgcnnnnnnttactggcactgatc

SEQ ID NO: 33 - DNA, 36 bp, Artificial Sequence; identical to SEQ ID NO: 32
  synthetic polynucleotide
  misc_feature (16)..(21): n = any nucleotide

SEQ ID NO: 34 - DNA, 36 bp, Artificial Sequence; identical to SEQ ID NO: 32
  synthetic polynucleotide
  misc_feature (16)..(21): n = any nucleotide

SEQ ID NO: 35 - DNA, 36 bp, Artificial Sequence; identical to SEQ ID NO: 32
  synthetic polynucleotide
  misc_feature (16)..(21): n = any nucleotide

SEQ ID NO: 36 - DNA, 36 bp, Artificial Sequence; identical to SEQ ID NO: 32
  synthetic polynucleotide
  misc_feature (16)..(21): n = any nucleotide

SEQ ID NO: 37 - DNA, 36 bp, Artificial Sequence; identical to SEQ ID NO: 32
  synthetic polynucleotide
  misc_feature (16)..(21): n = any nucleotide

SEQ ID NO: 38 - DNA, 36 bp, Artificial Sequence; identical to SEQ ID NO: 32
  synthetic polynucleotide
  misc_feature (16)..(21): n = any nucleotide

SEQ ID NO: 39 - DNA, 36 bp, Artificial Sequence; identical to SEQ ID NO: 32
  synthetic polynucleotide
  misc_feature (16)..(21): n = any nucleotide

SEQ ID NO: 40 - DNA, 36 bp, Artificial Sequence; identical to SEQ ID NO: 32
  synthetic polynucleotide
  misc_feature (16)..(21): n = any nucleotide

SEQ ID NO: 41 - DNA, 36 bp, Artificial Sequence
  synthetic polynucleotide
  misc_feature (16)..(21): n = any nucleotide
cgtacgcaatgacctnnnnnngcgcatttatgccat

SEQ ID NO: 42 - DNA, 36 bp, Artificial Sequence; identical to SEQ ID NO: 41
  synthetic polynucleotide
  misc_feature (16)..(21): n = any nucleotide

SEQ ID NO: 43 - DNA, 36 bp, Artificial Sequence; identical to SEQ ID NO: 41
  synthetic polynucleotide
  misc_feature (16)..(21): n = any nucleotide

SEQ ID NO: 44 - DNA, 36 bp, Artificial Sequence; identical to SEQ ID NO: 41
  synthetic polynucleotide
  misc_feature (16)..(21): n = any nucleotide

SEQ ID NO: 45 - DNA, 36 bp, Artificial Sequence; identical to SEQ ID NO: 41
  synthetic polynucleotide
  misc_feature (16)..(21): n = any nucleotide

SEQ ID NO: 46 - DNA, 36 bp, Artificial Sequence; identical to SEQ ID NO: 41
  synthetic polynucleotide
  misc_feature (16)..(21): n = any nucleotide

SEQ ID NO: 47 - DNA, 36 bp, Artificial Sequence; identical to SEQ ID NO: 41
  synthetic polynucleotide
  misc_feature (16)..(21): n = any nucleotide

SEQ ID NO: 48 - DNA, 36 bp, Artificial Sequence; identical to SEQ ID NO: 41
  synthetic polynucleotide
  misc_feature (16)..(21): n = any nucleotide

SEQ ID NO: 49 - DNA, 36 bp, Artificial Sequence; identical to SEQ ID NO: 41
  synthetic polynucleotide
  misc_feature (16)..(21): n = any nucleotide

SEQ ID NO: 50 - DNA, 36 bp, Artificial Sequence
  synthetic polynucleotide
  misc_feature (16)..(21): n = any nucleotide
gcatatcgcatcaagnnnnnncatggatcggtcatg

SEQ ID NO: 51 - DNA, 36 bp, Artificial Sequence; identical to SEQ ID NO: 50
  synthetic polynucleotide
  misc_feature (16)..(21): n = any nucleotide

SEQ ID NO: 52 - DNA, 36 bp, Artificial Sequence; identical to SEQ ID NO: 50
  synthetic polynucleotide
  misc_feature (16)..(21): n = any nucleotide

SEQ ID NO: 53 - DNA, 36 bp, Artificial Sequence; identical to SEQ ID NO: 50
  synthetic polynucleotide
  misc_feature (16)..(21): n = any nucleotide

SEQ ID NO: 54 - DNA, 36 bp, Artificial Sequence; identical to SEQ ID NO: 50
  synthetic polynucleotide
  misc_feature (16)..(21): n = any nucleotide

SEQ ID NO: 55 - DNA, 36 bp, Artificial Sequence; identical to SEQ ID NO: 50
  synthetic polynucleotide
  misc_feature (16)..(21): n = any nucleotide

SEQ ID NO: 56 - DNA, 36 bp, Artificial Sequence; identical to SEQ ID NO: 50
  synthetic polynucleotide
  misc_feature (16)..(21): n = any nucleotide

SEQ ID NO: 57 - DNA, 36 bp, Artificial Sequence; identical to SEQ ID NO: 50
  synthetic polynucleotide
  misc_feature (16)..(21): n = any nucleotide

SEQ ID NO: 58 - DNA, 36 bp, Artificial Sequence; identical to SEQ ID NO: 50
  synthetic polynucleotide
  misc_feature (16)..(21): n = any nucleotide

SEQ ID NO: 59 - DNA, 36 bp, Artificial Sequence
  synthetic polynucleotide
  misc_feature (16)..(27): n = any nucleotide
aatgaccgtgactatnnnnnnnnnnnnttttttttt

SEQ ID NO: 60 - DNA, 36 bp, Artificial Sequence; identical to SEQ ID NO: 59
  synthetic polynucleotide
  misc_feature (16)..(27): n = any nucleotide

SEQ ID NO: 61 - DNA, 36 bp, Artificial Sequence; identical to SEQ ID NO: 59
  synthetic polynucleotide
  misc_feature (16)..(27): n = any nucleotide

SEQ ID NO: 62 - DNA, 36 bp, Artificial Sequence; identical to SEQ ID NO: 59
  synthetic polynucleotide
  misc_feature (16)..(27): n = any nucleotide

SEQ ID NO: 63 - DNA, 36 bp, Artificial Sequence; identical to SEQ ID NO: 59
  synthetic polynucleotide
  misc_feature (16)..(27): n = any nucleotide

SEQ ID NO: 64 - DNA, 36 bp, Artificial Sequence; identical to SEQ ID NO: 59
  synthetic polynucleotide
  misc_feature (16)..(27): n = any nucleotide

SEQ ID NO: 65 - DNA, 36 bp, Artificial Sequence; identical to SEQ ID NO: 59
  synthetic polynucleotide
  misc_feature (16)..(27): n = any nucleotide

SEQ ID NO: 66 - DNA, 36 bp, Artificial Sequence; identical to SEQ ID NO: 59
  synthetic polynucleotide
  misc_feature (16)..(27): n = any nucleotide

SEQ ID NO: 67 - DNA, 36 bp, Artificial Sequence; identical to SEQ ID NO: 59
  synthetic polynucleotide
  misc_feature (16)..(27): n = any nucleotide

SEQ ID NO: 68 - DNA, 36 bp, Artificial Sequence
  synthetic polynucleotide
  misc_feature (16)..(27): n = any nucleotide
cgcgtaaatacggtannnnnnnnnnnnttttttttt

SEQ ID NO: 69 - DNA, 36 bp, Artificial Sequence; identical to SEQ ID NO: 68
  synthetic polynucleotide
  misc_feature (16)..(27): n = any nucleotide

SEQ ID NO: 70 - DNA, 36 bp, Artificial Sequence; identical to SEQ ID NO: 68
  synthetic polynucleotide
  misc_feature (16)..(27): n = any nucleotide

SEQ ID NO: 71 - DNA, 36 bp, Artificial Sequence; identical to SEQ ID NO: 68
  synthetic polynucleotide
  misc_feature (16)..(27): n = any nucleotide

SEQ ID NO: 72 - DNA, 36 bp, Artificial Sequence; identical to SEQ ID NO: 68
  synthetic polynucleotide
  misc_feature (16)..(27): n = any nucleotide

SEQ ID NO: 73 - DNA, 36 bp, Artificial Sequence; identical to SEQ ID NO: 68
  synthetic polynucleotide
  misc_feature (16)..(27): n = any nucleotide

SEQ ID NO: 74 - DNA, 36 bp, Artificial Sequence; identical to SEQ ID NO: 68
  synthetic polynucleotide
  misc_feature (16)..(27): n = any nucleotide

SEQ ID NO: 75 - DNA, 36 bp, Artificial Sequence; identical to SEQ ID NO: 68
  synthetic polynucleotide
  misc_feature (16)..(27): n = any nucleotide

SEQ ID NO: 76 - DNA, 36 bp, Artificial Sequence; identical to SEQ ID NO: 68
  synthetic polynucleotide
  misc_feature (16)..(27): n = any nucleotide

SEQ ID NO: 77 - DNA, 36 bp, Artificial Sequence
  synthetic polynucleotide
  misc_feature (16)..(27): n = any nucleotide
gtacctagccagtacnnnnnnnnnnnnttttttttt

SEQ ID NO: 78 - DNA, 36 bp, Artificial Sequence; identical to SEQ ID NO: 77
  synthetic polynucleotide
  misc_feature (16)..(27): n = any nucleotide

SEQ ID NO: 79 - DNA, 36 bp, Artificial Sequence; identical to SEQ ID NO: 77
  synthetic polynucleotide
  misc_feature (16)..(27): n = any nucleotide

SEQ ID NO: 80 - DNA, 36 bp, Artificial Sequence; identical to SEQ ID NO: 77
  synthetic polynucleotide
  misc_feature (16)..(27): n = any nucleotide

SEQ ID NO: 81 - DNA, 36 bp, Artificial Sequence; identical to SEQ ID NO: 77
  synthetic polynucleotide
  misc_feature (16)..(27): n = any nucleotide

SEQ ID NO: 82 - DNA, 36 bp, Artificial Sequence; identical to SEQ ID NO: 77
  synthetic polynucleotide
  misc_feature (16)..(27): n = any nucleotide

SEQ ID NO: 83 - DNA, 36 bp, Artificial Sequence; identical to SEQ ID NO: 77
  synthetic polynucleotide
  misc_feature (16)..(27): n = any nucleotide

SEQ ID NO: 84 - DNA, 36 bp, Artificial Sequence; identical to SEQ ID NO: 77
  synthetic polynucleotide
  misc_feature (16)..(27): n = any nucleotide

SEQ ID NO: 85 - DNA, 36 bp, Artificial Sequence; identical to SEQ ID NO: 77
  synthetic polynucleotide
  misc_feature (16)..(27): n = any nucleotide

SEQ ID NO: 86 - DNA, 79 bp, Artificial Sequence
  synthetic polynucleotide
  misc_feature (17)..(22): n = any nucleotide
  misc_feature (38)..(43): n = any nucleotide
  misc_feature (59)..(70): n = any nucleotide
tagttgcgtctcatgcnnnnnnatcgatagcgtaacgnnnnnnttactggcactgatcnnnnnnnnnnnnttttttttt

SEQ ID NO: 87 - DNA, 79 bp, Artificial Sequence; identical to SEQ ID NO: 86
  synthetic polynucleotide
  misc_feature (17)..(22): n = any nucleotide
  misc_feature (38)..(43): n = any nucleotide
  misc_feature (59)..(70): n = any nucleotide

SEQ ID NO: 88 - DNA, 37 bp, Artificial Sequence
  synthetic polynucleotide
  misc_feature (17)..(22): n = any nucleotide
tagttgcgtctcatgcnnnnnnatcgatagcgtaacg

SEQ ID NO: 89 - DNA, 37 bp, Artificial Sequence; identical to SEQ ID NO: 88
  synthetic polynucleotide
  misc_feature (17)..(22): n = any nucleotide

SEQ ID NO: 90 - DNA, 37 bp, Artificial Sequence; identical to SEQ ID NO: 88
  synthetic polynucleotide
  misc_feature (17)..(22): n = any nucleotide

SEQ ID NO: 91 - DNA, 37 bp, Artificial Sequence; identical to SEQ ID NO: 88
  synthetic polynucleotide
  misc_feature (17)..(22): n = any nucleotide

SEQ ID NO: 92 - DNA, 38 bp, Artificial Sequence
  synthetic polynucleotide
  misc_feature (17)..(22): n = any nucleotide
tagttgcgtctcatgcnnnnnngatcgatagcgtaacg

SEQ ID NO: 93 - DNA, 38 bp, Artificial Sequence; identical to SEQ ID NO: 92
  synthetic polynucleotide
  misc_feature (17)..(22): n = any nucleotide

SEQ ID NO: 94 - DNA, 39 bp, Artificial Sequence
  synthetic polynucleotide
  misc_feature (17)..(22): n = any nucleotide
tagttgcgtctcatgcnnnnnngcatcgatagcgtaacg

SEQ ID NO: 95 - DNA, 39 bp, Artificial Sequence; identical to SEQ ID NO: 94
  synthetic polynucleotide
  misc_feature (17)..(22): n = any nucleotide

SEQ ID NO: 96 - DNA, 39 bp, Artificial Sequence; identical to SEQ ID NO: 94
  synthetic polynucleotide
  misc_feature (17)..(22): n = any nucleotide

SEQ ID NO: 97 - DNA, 36 bp, Artificial Sequence; identical to SEQ ID NO: 32
  synthetic polynucleotide
  misc_feature (16)..(21): n = any nucleotide

SEQ ID NO: 98 - DNA, 36 bp, Artificial Sequence; identical to SEQ ID NO: 32
  synthetic polynucleotide
  misc_feature (16)..(21): n = any nucleotide

SEQ ID NO: 99 - DNA, 36 bp, Artificial Sequence; identical to SEQ ID NO: 32
  synthetic polynucleotide
  misc_feature (16)..(21): n = any nucleotide

SEQ ID NO: 100 - DNA, 36 bp, Artificial Sequence; identical to SEQ ID NO: 32
  synthetic polynucleotide
  misc_feature (16)..(21): n = any nucleotide

SEQ ID NO: 101 - DNA, 36 bp, Artificial Sequence; identical to SEQ ID NO: 32
  synthetic polynucleotide
  misc_feature (16)..(21): n = any nucleotide

SEQ ID NO: 102 - DNA, 36 bp, Artificial Sequence; identical to SEQ ID NO: 32
  synthetic polynucleotide
  misc_feature (16)..(21): n = any nucleotide

SEQ ID NO: 103 - DNA, 36 bp, Artificial Sequence; identical to SEQ ID NO: 32
  synthetic polynucleotide
  misc_feature (16)..(21): n = any nucleotide

SEQ ID NO: 104 - DNA, 36 bp, Artificial Sequence; identical to SEQ ID NO: 32
  synthetic polynucleotide
  misc_feature (16)..(21): n = any nucleotide

SEQ ID NO: 105 - DNA, 36 bp, Artificial Sequence; identical to SEQ ID NO: 32
  synthetic polynucleotide
  misc_feature (16)..(21): n = any nucleotide

SEQ ID NO: 106 - DNA, 36 bp, Artificial Sequence
  synthetic polynucleotide
  misc_feature (16)..(27): n = any nucleotide
aatgaccgtgactagnnnnnnnnnnnnttttttttt

SEQ ID NO: 107 - DNA, 36 bp, Artificial Sequence; identical to SEQ ID NO: 106
  synthetic polynucleotide
  misc_feature (16)..(27): n = any nucleotide

SEQ ID NO: 108 - DNA, 36 bp, Artificial Sequence; identical to SEQ ID NO: 106
  synthetic polynucleotide
  misc_feature (16)..(27): n = any nucleotide

SEQ ID NO: 109 - DNA, 36 bp, Artificial Sequence; identical to SEQ ID NO: 106
  synthetic polynucleotide
  misc_feature (16)..(27): n = any nucleotide

SEQ ID NO: 110 - DNA, 36 bp, Artificial Sequence; identical to SEQ ID NO: 106
  synthetic polynucleotide
  misc_feature (16)..(27): n = any nucleotide

SEQ ID NO: 111 - DNA, 36 bp, Artificial Sequence; identical to SEQ ID NO: 106
  synthetic polynucleotide
  misc_feature (16)..(27): n = any nucleotide

SEQ ID NO: 112 - DNA, 36 bp, Artificial Sequence; identical to SEQ ID NO: 106
  synthetic polynucleotide
  misc_feature (16)..(27): n = any nucleotide

SEQ ID NO: 113 - DNA, 36 bp, Artificial Sequence; identical to SEQ ID NO: 106
  synthetic polynucleotide
  misc_feature (16)..(27): n = any nucleotide

SEQ ID NO: 114 - DNA, 36 bp, Artificial Sequence; identical to SEQ ID NO: 106
  synthetic polynucleotide
  misc_feature (16)..(27): n = any nucleotide

SEQ ID NO: 115 - DNA, 79 bp, Artificial Sequence; identical to SEQ ID NO: 86
  synthetic polynucleotide
  misc_feature (17)..(22): n = any nucleotide
  misc_feature (38)..(43): n = any nucleotide
  misc_feature (59)..(70): n = any nucleotide

SEQ ID NO: 116 - DNA, 81 bp, Artificial Sequence
  synthetic polynucleotide
  misc_feature (17)..(22): n = any nucleotide
  misc_feature (40)..(45): n = any nucleotide
  misc_feature (61)..(72): n = any nucleotide
tagttgcgtctcatgcnnnnnngcatcgatagcgtaacgnnnnnnttactggcactgatcnnnnnnnnnnnnttttttttt

SEQ ID NO: 117 - DNA, 54 bp, Artificial Sequence
  synthetic polynucleotide
  misc_feature (13)..(18): n = any nucleotide
  misc_feature (34)..(39): n = any nucleotide
cgcagagtacgtnnnnnntagccatcgcattgcnnnnnntaccactgagctgaa

SEQ ID NO: 118 - DNA, 56 bp, Artificial Sequence
  synthetic polynucleotide
  misc_feature (25)..(32): n = any nucleotide
  misc_feature (36)..(41): n = any nucleotide
baaaaaaaaaaaaaaaaaaaacgtnnnnnnnncgtnnnnnnttcagctcagtggta